European Patent Specification EP 3 558 026 B1, published October 15, 2025. Title: Methods for Using Thermostable Proteases. Applicant: DuPont Nutrition Biosciences APS. The sequence listing filed with the application follows.

SEQUENCE LISTING (12 sequences)

SEQ ID NO: 1 - DNA, 1122 bp, Thermobifida cellulosilytica
gtgaaccgaccctccacccgcagaaccgtccgcgccctgctcaccgcggccctggcggccaccgcactgaccgccccggccgctccctccctcgcccaggaggcctcccaggaggccgccctcacccgcgacctcgacctgaccggaaccgaggtcgcgctgctgcgcgccgccgagtccgaggcgatggaccgcgaggaggagctgagcgccgtcctcggctccgacttcggcggcgtctacctggctccggagaccggagaggtcaccgtcgcggtcaccgaccccgcagccgtgcccgtcgtcgagcagtcgggggccaccgcccaggtcgtcaccttcggcgagaccgcgctcaacgacttcgtggactccctcaacgccgtcgccgaccgggccgacgagcagatcaccggctggtacaccgacctcgccgccgacacggtggtcatcaccgccttcccgggcggctccgctgccgccgaggagctggcggccctggcgggcgtcgacgaacgggcggtgcgggtcaccgagagcgccgcgcgaccgcaactgttcgccgacgtcatcggcggcaacccctactacttcggggggtaccgctgctccatcggcttctcggtgcgcaagggctcggacaccggcttcgccaccgccggccactgcggcgagacgggcaccctcacccgctcccccgagggcgtggtcgccggatcgtacttccccggacgcgacatgggctgggtgcgcctcaccggcgccgacaccgtcacccctctcgtcaaccgctacgacggggggaccgtgaccgtcaccggttcgcaggaggccgtcaccggctcctccgtctgccgctccggctccaccaccggctggcgctgcggcatcatccagtcgaagaaccagaccgtccgctacgccgagggcaccgtcaccggtctgacccgcaccaccgcctgcgccgaggccggcgactccggcggcccctggctcaccggctcccaggcccagggggtcacctcgggcggcagcggcaactgccggaccggcggcatcacctacttccagcccatcaacccgctgctgtcctacttcggcctggaactggtcaccggctga

SEQ ID NO: 2 - protein, 373 aa, Thermobifida cellulosilytica
MNRPSTRRTVRALLTAALAATALTAPAAPSLAQEASQEAALTRDLDLTGTEVALLRAAESEAMDREEELSAVLGSDFGGVYLAPETGEVTVAVTDPAAVPVVEQSGATAQVVTFGETALNDFVDSLNAVADRADEQITGWYTDLAADTVVITAFPGGSAAAEELAALAGVDERAVRVTESAARPQLFADVIGGNPYYFGGYRCSIGFSVRKGSDTGFATAGHCGETGTLTRSPEGVVAGSYFPGRDMGWVRLTGADTVTPLVNRYDGGTVTVTGSQEAVTGSSVCRSGSTTGWRCGIIQSKNQTVRYAEGTVTGLTRTTACAEAGDSGGPWLTGSQAQGVTSGGSGNCRTGGITYFQPINPLLSYFGLELVTG

SEQ ID NO: 3 - protein, 186 aa, Thermobifida cellulosilytica
ADVIGGNPYYFGGYRCSIGFSVRKGSDTGFATAGHCGETGTLTRSPEGVVAGSYFPGRDMGWVRLTGADTVTPLVNRYDGGTVTVTGSQEAVTGSSVCRSGSTTGWRCGIIQSKNQTVRYAEGTVTGLTRTTACAEAGDSGGPWLTGSQAQGVTSGGSGNCRTGGITYFQPINPLLSYFGLELVTG

SEQ ID NO: 4 - DNA, 1128 bp, artificial sequence
  codon-optimized DNA sequence encoding the pro-mature sequence of ME-3
gtgagaagcaaaaaattgtggatcagcttgttgtttgcgttaacgttaatctttacgatggcgttcagcaacatgtctgctagcgcagcaccgtcactggcacaagaagcatcacaagaagcagcactgacaagagatctggatctgacaggcacagaagttgcactgctgagagcagcagaatcagaagcaatggatagagaagaagaactgtcagcagttctgggctcagattttggcggagtttatctggcaccggaaacaggcgaagttacagttgcagttacagatccggcagcagttccggttgttgaacaatcaggcgcaacagcacaagttgttacatttggcgaaacagcgctgaatgattttgttgattcactgaatgcagttgcggatagagcagatgaacaaattacaggctggtatacagatcttgcagcagatacagttgtcattacagcatttccgggtggctcagcagcagcagaagaacttgcagcactggcaggcgttgatgaaagagcagttagagttacagaatcagcagcaagaccgcaactgtttgcagatgttattggcggaaatccgtattactttggcggatatagatgctcaattggcttttcagttagaaaaggctcagatacaggctttgcaacagcaggccattgcggagaaacaggcacactgacaagatcaccggaaggcgttgttgcaggctcatattttccgggaagagatatgggctgggttagactgacaggcgcagatacagtcacaccgctggttaatagatacgatggcggaacagttacagtcacaggcagccaagaagcagttacaggctcatcagtttgcagatcaggctcaacaacaggctggcgctgcggcattattcaatcaaaaaatcagacagttcgctatgcagaaggcacagttacaggcctgacaagaacaacagcatgcgcagaagcaggcgattcaggcggaccgtggctgacaggctcacaagcacaaggcgttacatcaggcggatcaggcaattgcagaacaggcggaattacatattttcagccgattaatccgctgctgtcatattttggcctggaactggttacaggctaa

SEQ ID NO: 5 - DNA, 93 bp, artificial sequence
  terminator
ggttaccttgaatgtatataaacattctcaaagggatttctaataaaaaacgctcggttgccgccgggcgttttttatgcatcgatggaattc

SEQ ID NO: 6 - DNA, 21 bp, artificial sequence
  linker
ggatcctgactgcctgagctt

SEQ ID NO: 7 - protein, 368 aa, Thermobifida fusca
MNHSSRRTTSLLFTAALAATALVAATTPASAQELALKRDLGLSDAEVAELRAAKAEAVELEEELRDSLGSDFGGVYLDADTTEITVAVTDPAAVSRVDADDVTVDVVDFGETALNDFVASLNAIADTADPKVTGWYTDLESDAVVITTLRGGTPAAEELAERAGLDERAVRIVEEDEEPQSLAAIIGGNPYYFGNYRCSIGFSVRQGSQTGFATAGHCGSTGTRVSSPSGTVAGSYFPGRDMGWVRITSADTVTPLVNRYNGGTVTVTGSQEAATGSSVCRSGATTGWRCGTIQSKNQTVRYAEGTVTGLTRTTACAEGGDSGGPWLTGSQAQGVTSGGTGDCRSGGITFFQPINPLLSYFGLQLVTG

SEQ ID NO: 8 - protein, 186 aa, Thermobifida fusca
AAIIGGNPYYFGNYRCSIGFSVRQGSQTGFATAGHCGSTGTRVSSPSGTVAGSYFPGRDMGWVRITSADTVTPLVNRYNGGTVTVTGSQEAATGSSVCRSGATTGWRCGTIQSKNQTVRYAEGTVTGLTRTTACAEGGDSGGPWLTGSQAQGVTSGGTGDCRSGGITFFQPINPLLSYFGLQLVTG

SEQ ID NO: 9 - protein, 353 aa, Thermobifida halotolerans
MVATALTASATPASADRHDALKRDLGLTDSEVARLRTAETEAMDREAELRDTLGSDFGGVHLDAASGELTIAVTDPEAVPTVERAGANAEVVTFGESALNGFVDSLNSVADQADEQVTGWYADIADDSVVITVREGGTAAAEALVARAGVDERAVRVTKSDERPQLFTDIIGGNPYYFDGYRCSIGFSVRRGSESGFATAGHCGEEGTETSDPEGTVAGAYFPGRDMGWVRITDADTVTPLVNRYNGENVTVAGSREAATGSSVCRSGSTTGWRCGTIRSKNQTVRYIEGTVTGLTRTTACAEGGDSGGPWLTGSQGQGVTSGGSGNCTLGGVTYFQPLNPLLSHFDLDLVTG

SEQ ID NO: 10 - protein, 186 aa, Thermobifida halotolerans
TDIIGGNPYYFDGYRCSIGFSVRRGSESGFATAGHCGEEGTETSDPEGTVAGAYFPGRDMGWVRITDADTVTPLVNRYNGENVTVAGSREAATGSSVCRSGSTTGWRCGTIRSKNQTVRYIEGTVTGLTRTTACAEGGDSGGPWLTGSQGQGVTSGGSGNCTLGGVTYFQPLNPLLSHFDLDLVTG

SEQ ID NO: 11 - protein, 375 aa, Nocardiopsis potens
MRKSPYISFLGASALALGMIAASPAAASADEAADTSPAEALASGLDMSASQAADLLDAEAEARGTEAEAREAAGGSFAGAVFDAESQVLTVSVTDAAAAEAVEATGAETRVVEASEDELDSAVSDLNAEESSLGSAIEGVTGWYVDPAANEVVVTVLDGETAAAETLLDEAGVDGVPVRIDEGAEQPETFGDIVGGNAYYPGGSRCSIGFSVQGGFATAGHCGSQGTRVTGGAGESGTVAGSIFPGRDMGWVRVNSGWNPSPYVNNYSGGRVLVTGSQEASVGASICRSGSTTGWHCGTIQAKNQTVRYPQGTVNGLTRTNVCAEPGDSGGSWISGSQAQGVTSGGSGNCSTGGTTFYQPINPILSQWGLTLTTG

SEQ ID NO: 12 - protein, 185 aa, Nocardiopsis potens
GDIVGGNAYYPGGSRCSIGFSVQGGFATAGHCGSQGTRVTGGAGESGTVAGSIFPGRDMGWVRVNSGWNPSPYVNNYSGGRVLVTGSQEASVGASICRSGSTTGWHCGTIQAKNQTVRYPQGTVNGLTRTNVCAEPGDSGGSWISGSQAQGVTSGGSGNCSTGGTTFYQPINPILSQWGLTLTTG